European Patent Application EP 4 306 543 A1, published January 17, 2024. Title: Anti ADAMTS13 antibody and the use thereof. Applicant: Nara Medical University National Institutes of Biomedical Innovation, Health and Nutrition Alfresa Pharma Corporation. The sequence listing filed with the application follows.

SEQUENCE LISTING (64 sequences)

SEQ ID NO: 1 - protein, 8 aa, Mus musculus
GYSFTGYT

SEQ ID NO: 2 - protein, 8 aa, Mus musculus
INPYNGGT

SEQ ID NO: 3 - protein, 10 aa, Mus musculus
ARTSGYLFAY

SEQ ID NO: 4 - protein, 6 aa, Mus musculus
EDIYNR

SEQ ID NO: 5 - protein, 3 aa, Mus musculus
GAT

SEQ ID NO: 6 - protein, 9 aa, Mus musculus
QQYWSSPLT

SEQ ID NO: 7 - protein, 8 aa, Mus musculus
GFSLPRYG

SEQ ID NO: 8 - protein, 7 aa, Mus musculus
IWAGGST

SEQ ID NO: 9 - protein, 11 aa, Mus musculus
ARAGGSQPFDY

SEQ ID NO: 10 - protein, 6 aa, Mus musculus
RDINTY

SEQ ID NO: 11 - protein, 3 aa, Mus musculus
RAN

SEQ ID NO: 12 - protein, 9 aa, Mus musculus
LQYDEFPWT

SEQ ID NO: 13 - protein, 8 aa, Mus musculus
GFSLTRYG

SEQ ID NO: 14 - protein, 7 aa, Mus musculus
IWAGGST

SEQ ID NO: 15 - protein, 11 aa, Mus musculus
ARAGGSSSFDY

SEQ ID NO: 16 - protein, 6 aa, Mus musculus
QDINTY

SEQ ID NO: 17 - protein, 3 aa, Mus musculus
RAN

SEQ ID NO: 18 - protein, 9 aa, Mus musculus
LQYDEFPWT

SEQ ID NO: 19 - protein, 8 aa, Mus musculus
GFSLTGYG

SEQ ID NO: 20 - protein, 7 aa, Mus musculus
IWADGTT

SEQ ID NO: 21 - protein, 11 aa, Mus musculus
ARAGGSQPFDY

SEQ ID NO: 22 - protein, 6 aa, Mus musculus
QDINSY

SEQ ID NO: 23 - protein, 3 aa, Mus musculus
RAN

SEQ ID NO: 24 - protein, 9 aa, Mus musculus
LQYDEFPWT

SEQ ID NO: 25 - protein, 117 aa, Mus musculus
EVQLQQSGPELVKPGTSMKISCKASGYSFTGYTMHWVKQSHGKNLEWIGLINPYNGGTGYNQKFKGKATLTVDKSSSTTYIELLSLTSEDSAVYYCARTSGYLFAYWGQGTLVTVSA

SEQ ID NO: 26 - protein, 107 aa, Mus musculus
DIQMTQSSSSFSVSLGDRVTITCKASEDIYNRLAWYQQKPGNAPRLLISGATSLETGVPSRFSGSGSGKDYIFSITSLQTEDVATYYCQQYWSSPLTFGAGTKLELK

SEQ ID NO: 27 - protein, 117 aa, Humanized
QIHLVESGGGVVQTGKSMKISCKASGYSFTGYTMHWVKQTPGKNLEWIGLINPYNGGTGYNQKFKGKATLTVDKSSSTTYIELLSLTSEDSAVYYCARTSGYLFAYWGQGTLVTVSS

SEQ ID NO: 28 - protein, 107 aa, Humanized
ETVMTQSPATLSVSPGERATITCKASEDIYNRLAWYQQKPGQAPRLLISGATSLETGVPSRFSGSGSGTEFTLTISSLQSEDVATYYCQQYWSSPLTFGAGTKLEIK

SEQ ID NO: 29 - protein, 117 aa, Humanized
QVQLVQSGGQVKKPGASVKISCKASGYSFTGYTMHWVKQAPGRGLEWIGLINPYNGGTGYNQKFKGKATLTVDKSSSTTYIELLSLTSEDSAVYYCARTSGYLFAYWGQGTLVTVSS

SEQ ID NO: 30 - protein, 107 aa, Humanized
DIVLTQTPDSLAVSLGERATITCKASEDIYNRLAWYQQKAGQPPKLLISGATSLETGVPDRFSGSGSGTDFTLTISSLQAEDVATYYCQQYWSSPLTFGAGTKVNIK

SEQ ID NO: 31 - protein, 117 aa, Mus musculus
QVQLRESGPGLVAPSQSLSITCTVSGFSLPRYGIHWVRQPPGKGLEWLGVIWAGGSTDYDSALMSRLSISKDTSKSQVFLKMSSLQTDDTAIYYCARAGGSQPFDYWGQGTTLTVSS

SEQ ID NO: 32 - protein, 107 aa, Mus musculus
DIKMTQSPSSMYASLGERVTITCKASRDINTYLSWFQQKPGKSPKTLISRANRLVDGVPSRFSGSGSGQDYSLSISSLEYEDMGFYYCLQYDEFPWTFGGGTKLVIK

SEQ ID NO: 33 - protein, 117 aa, Mus musculus
QVQLKESGPGLVAPSQSLSITCTVSGFSLTRYGVHWVRQPPGKGLEWLGVIWAGGSTNYKSALMSRLNITKDNSKSQVFLKMNGLQTDDTAIYFCARAGGSSSFDYWGQGTTLTVSS

SEQ ID NO: 34 - protein, 107 aa, Mus musculus
DIKMTQSPSSMNASLGERVTITCKASQDINTYLGWFQQKPGKSPKTLIYRANRLVDGVPSRFSGSGSGQGYSLTISSLEYEDMGIYYCLQYDEFPWTFGGGTKLEIK

SEQ ID NO: 35 - protein, 117 aa, Mus musculus
QVQLKESGPGLVAPSQSLSITCTVSGFSLTGYGIHWVRQPPGKGLEWLGVIWADGTTNSNSALMSRLSISKDNSKSQVFLKMTSLQTDDTAMYHCARAGGSQPFDYWGQGTTLTVSS

SEQ ID NO: 36 - protein, 107 aa, Mus musculus
DIKMTQSPSSMYASLGERVTITCKASQDINSYLSWFQQKPGKSPKTLIFRANRLVDGVPSRFSGSGSGQDYSLTISSLEYEDMEIYYCLQYDEFPWTFGGGTKLEIK

SEQ ID NO: 37 - protein, 488 aa, Humanized Chimera
MCPMSSPQTLNTLTPTMGWSWIFLFLLSGTAGVRSEVQLQQSGPELVKPGTSMKISCKASGYSFTGYTMHWVKQSHGKNLEWIGLINPYNGGTGYNQKFKGKATLTVDKSSSTTYIELLSLTSEDSAVYYCARTSGYLFAYWGQGTLVTVSAAKTTPPSVYPLAPGCGDTTGSSVTLGCLVKGYFPESVTVTWNSGSLSSSVHTFPALLQSGLYTMSSSVTVPSSTWPSQTVTCSVAHPASSTTVDKKLEPSGPISTINPCPPCKECHKCPAPNLEGGPSVFIFPPNIKDVLMISLTPKVTCVVVDVSEDDPDVQISWFVNNVEVHTAQTQTHREDYNSTIRVVSTLPIQHQDWMSGKEFKCKVNNKDLPSPIERTISKIKGLVRAPQVYILPPPAEQLSRKDVSLTCLVVGFNPGDISVEWTSNGHTEENYKDTAPVLDSDGSYFIYSKLNMKTSKWEKTDSFSCNVRHEGLKNYYLKKTISRSPGK

SEQ ID NO: 38 - protein, 241 aa, Humanized Chimera
MSGHSRNMKFPSQLLLLLLFGIPGMICDIQMTQSSSSFSVSLGDRVTITCKASEDIYNRLAWYQQKPGNAPRLLISGATSLETGVPSRFSGSGSGKDYIFSITSLQTEDVATYYCQQYWSSPLTFGAGTKLELKRADAAPTVSIFPPSSEQLTSGGASVVCFLNNFYPKDINVKWKIDGSERQNGVLNSWTDQDSKDSTYSMSSTLTLTKDEYERHNSYTCEATHKTSTSPILKSFNRNEC

SEQ ID NO: 39 - protein, 447 aa, Humanized
QIHLVESGGGVVQTGKSMKISCKASGYSFTGYTMHWVKQTPGKNLEWIGLINPYNGGTGYNQKFKGKATLTVDKSSSTTYIELLSLTSEDSAVYYCARTSGYLFAYWGQGTLVTVSSASTKGPSVFPLAPSSKSTSGGTAALGCLVRDYFPEPVTVSWNSGALTSGVHTFPAVLQSSGLYSLSSVVTVPSSSLGTQTYICNVNHKPSNTKVDKKVEPKSCDKTHTCPPCPAPELLGGPSVFLFPPKPKDTLMISRTPEVTCVVVDVSHEDPEVKFNWYVDGVEVHNAKTKPREEQYNSTYRVVSVLTVVHQDWLNGKEYKCKVSNKALPAPIEKTISKAKGQPREPQVYTLPPSRDELTKNQVSLTCLVKGFYPSDIAVEWESNGQPENNYKTTPPVLDSDGSFFLYSKLTVDKSRWQQGNVFSCSVMHEALHNHYTQKSLSLSPGK

SEQ ID NO: 40 - protein, 214 aa, Humanized
ETVMTQSPATLSVSPGERATITCKASEDIYNRLAWYQQKPGQAPRLLISGATSLETGVPSRFSGSGSGTEFTLTISSLQSEDVATYYCQQYWSSPLTFGAGTKLEIKRTVAAPSVFIFPPSDEQLKSGTASVVCLLNNFYPREAKVQWKVDNALQSGNSQESVTEQDSKDSTYSLSSTLTLSKADYEKHKVYACEVTHQGLSSPVTKSFNRGEC

SEQ ID NO: 41 - protein, 447 aa, Humanized
QVQLVQSGGQVKKPGASVKISCKASGYSFTGYTMHWVKQAPGRGLEWIGLINPYNGGTGYNQKFKGKATLTVDKSSSTTYIELLSLTSEDSAVYYCARTSGYLFAYWGQGTLVTVSSASTKGPSVFPLAPSSKSTSGGTAALGCLVKDYFPEPVTVSWNSGALTSGVHTFPAVLQSSGLYSLSSVVTVPSSSLGTQTYICNVNHKPSNTKVDKKVEPKSCDKTHTCPPCPAPELLGGPSVFLFPPKPKDTLMISRTPEVTCVVVDVSHEDPEVKFNWYVDGVEVHNAKTKPREEQYNSTYRVVSVLTVLHQDWLNGKEYKCKVSNKALPAPIEKTISKAKGQPREPQVYTLPPSRDELTKNQVSLTCLVKGFYPSDIAVEWESNGQPENNYKTTPPVLDSDGSFFLYSKLTVDKSRWQQGNIFSCSVMHEALHNHYTQKSLSLSPGK

SEQ ID NO: 42 - protein, 214 aa, Humanized
DIVLTQTPDSLAVSLGERATITCKASEDIYNRLAWYQQKAGQPPKLLISGATSLETGVPDRFSGSGSGTDFTLTISSLQAEDVATYYCQQYWSSPLTFGAGTKVNIKRTVAAPSVFIFPPSDEQLKSGTASVVCLLNNFYPREAKVQWKVDNALQSGNSQESVTEQDSKDSTYSLSSTLTLSKADYEKHKVYACEVTHQGLSSPVTKSFNRGEC

SEQ ID NO: 43 - protein, 460 aa, Mus musculus
MAVLVLFLCLVAFPSCVLSQVQLRESGPGLVAPSQSLSITCTVSGFSLPRYGIHWVRQPPGKGLEWLGVIWAGGSTDYDSALMSRLSISKDTSKSQVFLKMSSLQTDDTAIYYCARAGGSQPFDYWGQGTTLTVSSAKTTPPSVYPLAPGSAAQTNSMVTLGCLVKGYFPEPVTVTWNSGSLSSGVHTFPAVLQSDLYTLSSSVTVPSSTWPSETVTCNVAHPASSTKVDKKIVPRDCGCKPCICTVPEVSSVFIFPPKPKDVLTITLTPKVTCVVVDISKDDPEVQFSWFVDDVEVHTAQTQPREEQFNSTFRSVSELPIMHQDWLNGKEFKCRVNSAAFPAPIEKTISKTKGRPKAPQVYTIPPPKEQMAKDKVSLTCMITDFFPEDITVEWQWNGQPAENYKNTQPIMDTDGSYFVYSKLNVQKSNWEAGNTFTCSVLHEGLHNHHTEKSLSHSPGK

SEQ ID NO: 44 - protein, 236 aa, Mus musculus
MDMRTPAQFLGILLLWFPGIKCDIKMTQSPSSMYASLGERVTITCKASRDINTYLSWFQQKPGKSPKTLISRANRLVDGVPSRFSGSGSGQDYSLSISSLEYEDMGFYYCLQYDEFPWTFGGGTKLVIKRADAAPTVSIFPPSSEQLTSGGASVVCFLNNFYPKDINVKWKIDGSERQNGVLNSWTDQDSKDSTYSMSSTLTLTKDEYERHNSYTCEATHKTSTSPIVKSFNRNEW

SEQ ID NO: 45 - protein, 460 aa, Mus musculus
MAVLVLFLCLVAFPSCVLSQVQLKESGPGLVAPSQSLSITCTVSGFSLTRYGVHWVRQPPGKGLEWLGVIWAGGSTNYKSALMSRLNITKDNSKSQVFLKMNGLQTDDTAIYFCARAGGSSSFDYWGQGTTLTVSSAKTTPPSVYPLAPGSAAQTNSMVTLGCLVKGYFPEPVTVTWNSGSLSSGVHTFPAVLQSDLYTLSSSVTVPSSTWPSETVTCNVAHPASSTKVDKKIVPRDCGCKPCICTVPEVSSVFIFPPKPKDVLTITLTPKVTCVVVDISKDDPEVQFSWFVDDVEVHTAQTQPREEQFNSTFRSVSELPIMHQDWLNGKEFKCRVNSAAFPAPIEKTISKTKGRPKAPQVYTIPPPKEQMAKDKVSLTCMITDFFPEDITVEWQWNGQPAENYKNTQPIMDTDGSYFVYSKLNVQKSNWEAGNTFTCSVLHEGLHNHHTEKSLSHSPGK

SEQ ID NO: 46 - protein, 236 aa, Mus musculus
MDMRTPAQFLGILLLWFPGIKCDIKMTQSPSSMNASLGERVTITCKASQDINTYLGWFQQKPGKSPKTLIYRANRLVDGVPSRFSGSGSGQGYSLTISSLEYEDMGIYYCLQYDEFPWTFGGGTKLEIKRADAAPTVSIFPPSSEQLTSGGASVVCFLNNFYPKDINVKWKIDGSERQNGVLNSWTDQDSKDSTYSMSSTLTLTKDEYERHNSYTCEATHKTSTSPIVKSFNRNEC

SEQ ID NO: 47 - protein, 472 aa, Mus musculus
MAVLVLFLCLVAFPSCVLSQVQLKESGPGLVAPSQSLSITCTVSGFSLTGYGIHWVRQPPGKGLEWLGVIWADGTTNSNSALMSRLSISKDNSKSQVFLKMTSLQTDDTAMYHCARAGGSQPFDYWGQGTTLTVSSAKTTPPSVYPLAPGCGDTTGSSVTLGCLVKGYFPESVTVTWNSGSLSSSVHTFPALLQSGLYTMSSSVTVPSSTWPSQTVTCSVAHPASSTTVDKKLEPSGPISTINPCPPCKECHKCPAPNLEGGPSVFIFPPNIKDVLMISLTPKVTCVVVDVSEDDPDVQISWFVNNVEVHTAQTQTHREDYNSTIRVVSTLPIQHQDWMSGKEFKCKVNNKDLPSPIERTISKIKGLVRAPQVYILPPPAEQLSRKDVSLTCLVVGFNPGDISVEWTSNGHTEENYKDTAPVLDSDGSYFIYSKLNMKTSKWEKTDSFSCNVRHEGLKNYYLKKTISRSPGK

SEQ ID NO: 48 - protein, 234 aa, Mus musculus
MRTPAQFLGILLLWFPGIKCDIKMTQSPSSMYASLGERVTITCKASQDINSYLSWFQQKPGKSPKTLIFRANRLVDGVPSRFSGSGSGQDYSLTISSLEYEDMEIYYCLQYDEFPWTFGGGTKLEIKRADAAPTVSIFPPSSEQLTSGGASVVCFLNNFYPKDINVKWKIDGSERQNGVLNSWTDQDSKDSTYSMSSTLTLTKDEYERHNSYTCEATHKTSTSPIVKSFNRNEW

SEQ ID NO: 49 - DNA, 23 bp, Artificial Sequence
  Forward primer for A10 ab
aagcagtggtatcaacgcagagt

SEQ ID NO: 50 - DNA, 30 bp, Artificial Sequence
  Reverse primer for A10 ab and 9A7 ab
taggacctgagagctttgtgggtgctgagc

SEQ ID NO: 51 - DNA, 32 bp, Artificial Sequence
  Forward primer for A10 ab
ggggcggccgcagagtggccattacggccggg

SEQ ID NO: 52 - DNA, 35 bp, Artificial Sequence
  Reverse primer for A10 ab and 9A7 ab
ggggaattctcatttacccggagaccgggagatgg

SEQ ID NO: 53 - DNA, 20 bp, Artificial Sequence
  Forward primer for A10 ab CH
gcctccaccaagggcccatc

SEQ ID NO: 54 - DNA, 20 bp, Artificial Sequence
  Reverse primer for A10 ab CH
gcggccgcggtcaccaattc

SEQ ID NO: 55 - DNA, 36 bp, Artificial Sequence
  Forward primer for A10 ab VH
gaattggtgaccgcggccgcagagtggccattacgg

SEQ ID NO: 56 - DNA, 36 bp, Artificial Sequence
  Reverse primer for A10 ab VH
gggcccttggtggaggctgcagagacagtgaccaga

SEQ ID NO: 57 - DNA, 20 bp, Artificial Sequence
  Forward primer for A10 ab CL
cgaactgtggctgcaccatc

SEQ ID NO: 58 - DNA, 20 bp, Artificial Sequence
  Reverse primer for A10 ab CL
gcggccgcggtcaccaattc

SEQ ID NO: 59 - DNA, 36 bp, Artificial Sequence; identical to SEQ ID NO: 55
  Forward primer for A10 ab VL

SEQ ID NO: 60 - DNA, 41 bp, Artificial Sequence
  Reverse primer for A10 ab VL
gatggtgcagccacagttcgtttcagctccagcttggtccc

SEQ ID NO: 61 - DNA, 23 bp, Artificial Sequence
  Forward primer for  1G2 ab, 12D10 ab, 9A7 ab
aagcagtggtatcaacgcagagt

SEQ ID NO: 62 - DNA, 30 bp, Artificial Sequence
  Reverse primer for  1G2 ab, 12D10 ab
taggaccagagggctccaaggacactggga

SEQ ID NO: 63 - DNA, 32 bp, Artificial Sequence; identical to SEQ ID NO: 51
  Forward primer for  1G2 ab, 12D10 ab, 9A7 ab

SEQ ID NO: 64 - DNA, 35 bp, Artificial Sequence
  Reverse primer for  1G2 ab, 12D10 ab
ggggaattctcatttaccaggagagtgggagaggc